European Patent Specification EP 4 358 995 B1, published December 3, 2025. Title: THERAPIES FOR WEIGHT MANAGEMENT AND RELATED METABOLIC CONDITIONS. Applicant: SCHOLAR ROCK, INC. The sequence listing filed with the application follows.

SEQUENCE LISTING (133 sequences)

SEQ ID NO: 1 - protein, 6 aa, Artificial Sequence
  Description of Artificial Sequence: Synthetic peptide
SSYGMH

SEQ ID NO: 2 - protein, 10 aa, Artificial Sequence
  Description of Artificial Sequence: Synthetic peptide
GFTFSSYGMH

SEQ ID NO: 3 - protein, 10 aa, Artificial Sequence
  Description of Artificial Sequence: Synthetic peptide
GFAFSSYGMH

SEQ ID NO: 4 - protein, 17 aa, Artificial Sequence
  Description of Artificial Sequence: Synthetic peptide
VISYDGSNKYYADSVKG

SEQ ID NO: 5 - protein, 7 aa, Artificial Sequence
  Description of Artificial Sequence: Synthetic peptide
ISYDGSN

SEQ ID NO: 6 - protein, 17 aa, Artificial Sequence
  Description of Artificial Sequence: Synthetic peptide
VISYDGSIKYYADSVKG

SEQ ID NO: 7 - protein, 7 aa, Artificial Sequence
  Description of Artificial Sequence: Synthetic peptide
ISYDGSI

SEQ ID NO: 8 - protein, 17 aa, Artificial Sequence
  Description of Artificial Sequence: Synthetic peptide
VISYDGNNKYYADSVKG

SEQ ID NO: 9 - protein, 7 aa, Artificial Sequence
  Description of Artificial Sequence: Synthetic peptide
ISYDGNN

SEQ ID NO: 10 - protein, 17 aa, Artificial Sequence
  Description of Artificial Sequence: Synthetic peptide
DLLVRFLEWSHYYGMDV

SEQ ID NO: 11 - protein, 17 aa, Artificial Sequence
  Description of Artificial Sequence: Synthetic peptide
DLLVRFLEWSHKYGMDV

SEQ ID NO: 12 - protein, 13 aa, Artificial Sequence
  Description of Artificial Sequence: Synthetic peptide
SGSSSNIGSNTVH

SEQ ID NO: 13 - protein, 8 aa, Artificial Sequence
  Description of Artificial Sequence: Synthetic peptide
SSNIGSNT

SEQ ID NO: 14 - protein, 13 aa, Artificial Sequence
  Description of Artificial Sequence: Synthetic peptide
SGSTSNIGSNTVH

SEQ ID NO: 15 - protein, 8 aa, Artificial Sequence
  Description of Artificial Sequence: Synthetic peptide
TSNIGSNT

SEQ ID NO: 16 - protein, 13 aa, Artificial Sequence
  Description of Artificial Sequence: Synthetic peptide
SGSSSNIGGNTVH

SEQ ID NO: 17 - protein, 5 aa, Artificial Sequence
  Description of Artificial Sequence: Synthetic peptide
  MOD_RES (1)..(2): Any amino acid
XXDIS

SEQ ID NO: 18 - protein, 16 aa, Artificial Sequence
  Description of Artificial Sequence: Synthetic peptide
IISYAGSTYYASWAKG

SEQ ID NO: 19 - protein, 11 aa, Artificial Sequence
  Description of Artificial Sequence: Synthetic peptide
  MOD_RES (7)..(7): Any amino acid
GVPAYSXGGDL

SEQ ID NO: 20 - protein, 13 aa, Artificial Sequence
  Description of Artificial Sequence: Synthetic peptide
  MOD_RES (1)..(2): Any amino acid
  MOD_RES (8)..(9): Any amino acid
XXSQSVYXXNWLS

SEQ ID NO: 21 - protein, 7 aa, Artificial Sequence
  Description of Artificial Sequence: Synthetic peptide
  MOD_RES (7)..(7): Any amino acid
WASTLAX

SEQ ID NO: 22 - protein, 10 aa, Artificial Sequence
  Description of Artificial Sequence: Synthetic peptide
  MOD_RES (8)..(8): Any amino acid
AGGYGGGXYA

SEQ ID NO: 23 - protein, 10 aa, Artificial Sequence
  Description of Artificial Sequence: Synthetic peptide
AAWDESLNGV

SEQ ID NO: 24 - protein, 126 aa, Artificial Sequence
  Description of Artificial Sequence: Synthetic polypeptide
QIQLVQSGGGVVQPGRSLRLSCAASGFTFSSYGMHWVRQAPGKGLEWVAVISYDGSNKYYADSVKGRFTISRDNSKNTLYLQMNSLRAEDTAVYYCARDLLVRFLEWSHYYGMDVWGQGTTVTVSS

SEQ ID NO: 25 - protein, 126 aa, Artificial Sequence
  Description of Artificial Sequence: Synthetic polypeptide
QVQLVESGGGVVQPGRSLRLSCAASGFTFSSYGMHWVRQAPGKGLEWVAVISYDGSNKYYADSVKGRFTISRDNSKNTLYLQMNSLRAEDTAVYYCARDLLVRFLEWSHYYGMDVWGQGTTVTVSS

SEQ ID NO: 26 - protein, 126 aa, Artificial Sequence
  Description of Artificial Sequence: Synthetic polypeptide
QIQLVQSGGGVVQPGRSLRLSCAASGFAFSSYGMHWVRQAPGKGLEWVAVISYDGSIKYYADSVKGRFTISRDNSKNTLYLQMNSLRAEDTAVYYCARDLLVRFLEWSHKYGMDVWGQGTTVTVSS

SEQ ID NO: 27 - protein, 126 aa, Artificial Sequence
  Description of Artificial Sequence: Synthetic polypeptide
QVQLVESGGGVVQPGRSLRLSCAASGFAFSSYGMHWVRQAPGKGLEWVAVISYDGSIKYYADSVKGRFTISRDNSKNTLYLQMNSLRAEDTAVYYCARDLLVRFLEWSHKYGMDVWGQGTTVTVSS

SEQ ID NO: 28 - protein, 126 aa, Artificial Sequence
  Description of Artificial Sequence: Synthetic polypeptide
QIQLVQSGGGVVQPGRSLRLSCAASGFAFSSYGMHWVRQAPGKGLEWVAVISYDGNNKYYADSVKGRFTISRDNSKNTLYLQMNSLRAEDTAVYYCARDLLVRFLEWSHKYGMDVWGQGTTVTVSS

SEQ ID NO: 29 - protein, 126 aa, Artificial Sequence
  Description of Artificial Sequence: Synthetic polypeptide
QVQLVESGGGVVQPGRSLRLSCAASGFAFSSYGMHWVRQAPGKGLEWVAVISYDGNNKYYADSVKGRFTISRDNSKNTLYLQMNSLRAEDTAVYYCARDLLVRFLEWSHKYGMDVWGQGTTVTVSS

SEQ ID NO: 30 - protein, 109 aa, Artificial Sequence
  Description of Artificial Sequence: Synthetic polypeptide
QPVLTQPPSASGTPGQRVTISCSGSSSNIGSNTVHWYQQLPGTAPKLLIYSDNQRPSGVPDRFSGSKSGTSASLVISGLQSDDEADYYCAAWDDSLNGVFGGGTKLTVL

SEQ ID NO: 31 - protein, 109 aa, Artificial Sequence
  Description of Artificial Sequence: Synthetic polypeptide
QSVLTQPPSASGTPGQRVTISCSGSSSNIGSNTVHWYQQLPGTAPKLLIYSDNQRPSGVPDRFSGSKSGTSASLAISGLQSEDEADYYCAAWDDSLNGVFGGGTKLTVL

SEQ ID NO: 32 - protein, 109 aa, Artificial Sequence
  Description of Artificial Sequence: Synthetic polypeptide
QPVLTQPPSASGTPGQRVTISCSGSTSNIGSNTVHWYQQLPGTAPKLLIYSDDQRPSGVPDRFSGSKSGTSASLVISGLQSDDEADYYCAAWDESLNGVFGGGTKLTVL

SEQ ID NO: 33 - protein, 109 aa, Artificial Sequence
  Description of Artificial Sequence: Synthetic polypeptide
QSVLTQPPSASGTPGQRVTISCSGSTSNIGSNTVHWYQQLPGTAPKLLIYSDDQRPSGVPDRFSGSKSGTSASLAISGLQSEDEADYYCAAWDESLNGVFGGGTKLTVL

SEQ ID NO: 34 - protein, 109 aa, Artificial Sequence
  Description of Artificial Sequence: Synthetic polypeptide
QPVLTQPPSASGTPGQRVTISCSGSSSNIGGNTVHWYQQLPGTAPKLLIYSDDQRPSGVPDRFSGSKSGTSASLVISGLQSDDEADYYCAAWDESLNGVFGGGTKLTVL

SEQ ID NO: 35 - protein, 109 aa, Artificial Sequence
  Description of Artificial Sequence: Synthetic polypeptide
QSVLTQPPSASGTPGQRVTISCSGSSSNIGGNTVHWYQQLPGTAPKLLIYSDDQRPSGVPDRFSGSKSGTSASLAISGLQSEDEADYYCAAWDESLNGVFGGGTKLTVL

SEQ ID NO: 36 - protein, 98 aa, Artificial Sequence
  Description of Artificial Sequence: Synthetic polypeptide
QVQLVESGGGVVQPGRSLRLSCAASGFTFSSYGMHWVRQAPGKGLEWVAVISYDGSNKYYADSVKGRFTISRDNSKNTLYLQMNSLRAEDTAVYYCAR

SEQ ID NO: 37 - protein, 98 aa, Artificial Sequence
  Description of Artificial Sequence: Synthetic polypeptide
QSVLTQPPSASGTPGQRVTISCSGSSSNIGSNTVNWYQQLPGTAPKLLIYSNNQRPSGVPDRFSGSKSGTSASLAISGLQSEDEADYYCAAWDDSLNG

SEQ ID NO: 38 - DNA, 378 bp, Artificial Sequence
  Description of Artificial Sequence: Synthetic polynucleotide
cagatccagctggtgcagtctgggggaggcgtggtccagcctgggaggtccctgagactctcctgtgcagcgtctggattcaccttcagtagctatggcatgcactgggtccgccaggctccaggcaaggggctggagtgggtggcagttatatcatatgatggaagtaataaatactatgcagactccgtgaagggccgattcaccatctccagagacaattccaagaacacgctgtatctgcaaatgaacagcctgagagccgaggacacggctgtgtattactgtgcgagagatctcctggtgcgatttttggagtggtcgcactactacggtatggacgtctggggccaagggaccacggtcaccgtctcctca

SEQ ID NO: 39 - DNA, 378 bp, Artificial Sequence
  Description of Artificial Sequence: Synthetic polynucleotide
caggtgcagctggtggagtctgggggaggcgtggtccagcctgggaggtccctgagactctcctgtgcagcgtctggattcaccttcagtagctatggcatgcactgggtccgccaggctccaggcaaggggctggagtgggtggcagttatatcatatgatggaagtaataaatactatgcagactccgtgaagggccgattcaccatctccagagacaattccaagaacacgctgtatctgcaaatgaacagcctgagagccgaggacacggctgtgtattactgtgcgagagatctcctggtgcgatttttggagtggtcgcactactacggtatggacgtctggggccaagggaccacggtcaccgtctcctca

SEQ ID NO: 40 - DNA, 378 bp, Artificial Sequence
  Description of Artificial Sequence: Synthetic polynucleotide
cagatccagctggtgcagtctgggggaggcgtggtccagcctgggaggtccctgagactctcctgtgcagcgtctggattcgccttcagtagctatggcatgcactgggtccgccaggctccaggcaaggggctggagtgggtggcagttatatcatatgatggaagtatcaaatactatgcagactccgtgaagggccgattcaccatctccagagacaattccaagaacacgctgtatctgcaaatgaacagcctgagagccgaggacacggctgtgtattactgtgcgagagatctcctggtgcgatttttggagtggtcgcacaagtacggtatggacgtctggggccaagggaccacggtcaccgtctcctca

SEQ ID NO: 41 - DNA, 378 bp, Artificial Sequence
  Description of Artificial Sequence: Synthetic polynucleotide
caggtgcagctggtggagtctgggggaggcgtggtccagcctgggaggtccctgagactctcctgtgcagcgtctggattcgccttcagtagctatggcatgcactgggtccgccaggctccaggcaaggggctggagtgggtggcagttatatcatatgatggaagtatcaaatactatgcagactccgtgaagggccgattcaccatctccagagacaattccaagaacacgctgtatctgcaaatgaacagcctgagagccgaggacacggctgtgtattactgtgcgagagatctcctggtgcgatttttggagtggtcgcacaagtacggtatggacgtctggggccaagggaccacggtcaccgtctcctca

SEQ ID NO: 42 - DNA, 378 bp, Artificial Sequence
  Description of Artificial Sequence: Synthetic polynucleotide
cagatccagctggtgcagtctgggggaggcgtggtccagcctgggaggtccctgagactctcctgtgcagcgtctggattcgccttcagtagctatggcatgcactgggtccgccaggctccaggcaaggggctggagtgggtggcagttatatcatatgatggaaataataaatactatgcagactccgtgaagggccgattcaccatctccagagacaattccaagaacacgctgtatctgcaaatgaacagcctgagagccgaggacacggctgtgtattactgtgcgagagatctcctggtgcgatttttggagtggtcgcacaagtacggtatggacgtctggggccaagggaccacggtcaccgtctcctca

SEQ ID NO: 43 - DNA, 378 bp, Artificial Sequence
  Description of Artificial Sequence: Synthetic polynucleotide
caggtgcagctggtggagtctgggggaggcgtggtccagcctgggaggtccctgagactctcctgtgcagcgtctggattcgccttcagtagctatggcatgcactgggtccgccaggctccaggcaaggggctggagtgggtggcagttatatcatatgatggaaataataaatactatgcagactccgtgaagggccgattcaccatctccagagacaattccaagaacacgctgtatctgcaaatgaacagcctgagagccgaggacacggctgtgtattactgtgcgagagatctcctggtgcgatttttggagtggtcgcacaagtacggtatggacgtctggggccaagggaccacggtcaccgtctcctca

SEQ ID NO: 44 - DNA, 327 bp, Artificial Sequence
  Description of Artificial Sequence: Synthetic polynucleotide
cagcctgtgctgactcagccaccctcagcgtctgggacccccgggcagagggtcaccatctcttgttctggaagcagctccaacatcggaagtaatactgtccactggtaccagcaactcccaggaacggcccccaaactcctcatctatagtgataatcagcgcccctcaggggtccctgaccgattctctggctccaagtctggcacctcagcctccctggtcatcagtgggctccagtctgacgatgaggctgattattactgtgcagcatgggatgacagcctgaatggggtgttcggcggagggaccaagctgaccgtccta

SEQ ID NO: 45 - DNA, 327 bp, Artificial Sequence
  Description of Artificial Sequence: Synthetic polynucleotide
cagtctgtgctgactcagccaccctcagcgtctgggacccccgggcagagggtcaccatctcttgttctggaagcagctccaacatcggaagtaatactgtccactggtaccagcaactcccaggaacggcccccaaactcctcatctatagtgataatcagcgcccctcaggggtccctgaccgattctctggctccaagtctggcacctcagcctccctggccatcagtgggctccagtctgaggatgaggctgattattactgtgcagcatgggatgacagcctgaatggggtgttcggcggagggaccaagctgaccgtccta

SEQ ID NO: 46 - DNA, 327 bp, Artificial Sequence
  Description of Artificial Sequence: Synthetic polynucleotide
cagcctgtgctgactcagccaccctcagcgtctgggacccccgggcagagggtcaccatctcttgttctggaagcacctccaacatcggaagtaatactgtccactggtaccagcaactcccaggaacggcccccaaactcctcatctatagtgatgatcagcgcccctcaggggtccctgaccgattctctggctccaagtctggcacctcagcctccctggtcatcagtgggctccagtctgacgatgaggctgattattactgtgcagcatgggatgagagcctgaatggggtgttcggcggagggaccaagctgaccgtccta

SEQ ID NO: 47 - DNA, 327 bp, Artificial Sequence
  Description of Artificial Sequence: Synthetic polynucleotide
cagtctgtgctgactcagccaccctcagcgtctgggacccccgggcagagggtcaccatctcttgttctggaagcacctccaacatcggaagtaatactgtccactggtaccagcaactcccaggaacggcccccaaactcctcatctatagtgatgatcagcgcccctcaggggtccctgaccgattctctggctccaagtctggcacctcagcctccctggccatcagtgggctccagtctgaggatgaggctgattattactgtgcagcatgggatgagagcctgaatggggtgttcggcggagggaccaagctgaccgtccta

SEQ ID NO: 48 - DNA, 327 bp, Artificial Sequence
  Description of Artificial Sequence: Synthetic polynucleotide
cagcctgtgctgactcagccaccctcagcgtctgggacccccgggcagagggtcaccatctcttgttctggaagcagctccaacatcggaggaaatactgtccactggtaccagcaactcccaggaacggcccccaaactcctcatctatagtgatgatcagcgcccctcaggggtccctgaccgattctctggctccaagtctggcacctcagcctccctggtcatcagtgggctccagtctgacgatgaggctgattattactgtgcagcatgggatgagagcctgaatggggtgttcggcggagggaccaagctgaccgtccta

SEQ ID NO: 49 - DNA, 327 bp, Artificial Sequence
  Description of Artificial Sequence: Synthetic polynucleotide
cagtctgtgctgactcagccaccctcagcgtctgggacccccgggcagagggtcaccatctcttgttctggaagcagctccaacatcggaggaaatactgtccactggtaccagcaactcccaggaacggcccccaaactcctcatctatagtgatgatcagcgcccctcaggggtccctgaccgattctctggctccaagtctggcacctcagcctccctggccatcagtgggctccagtctgaggatgaggctgattattactgtgcagcatgggatgagagcctgaatggggtgttcggcggagggaccaagctgaccgtccta

SEQ ID NO: 50 - protein, 452 aa, Artificial Sequence
  Description of Artificial Sequence: Synthetic polypeptide
QVQLVESGGGVVQPGRSLRLSCAASGFTFSSYGMHWVRQAPGKGLEWVAVISYDGSNKYYADSVKGRFTISRDNSKNTLYLQMNSLRAEDTAVYYCARDLLVRFLEWSHYYGMDVWGQGTTVTVSSASTKGPSVFPLAPCSRSTSESTAALGCLVKDYFPEPVTVSWNSGALTSGVHTFPAVLQSSGLYSLSSVVTVPSSSLGTKTYTCNVDHKPSNTKVDKRVESKYGPPCPPCPAPEFLGGPSVFLFPPKPKDTLMISRTPEVTCVVVDVSQEDPEVQFNWYVDGVEVHNAKTKPREEQFNSTYRVVSVLTVLHQDWLNGKEYKCKVSNKGLPSSIEKTISKAKGQPREPQVYTLPPSQEEMTKNQVSLTCLVKGFYPSDIAVEWESNGQPENNYKTTPPVLDSDGSFFLYSRLTVDKSRWQEGNVFSCSVMHEALHNHYTQKSLSLSLG

SEQ ID NO: 51 - protein, 215 aa, Artificial Sequence
  Description of Artificial Sequence: Synthetic polypeptide
QSVLTQPPSASGTPGQRVTISCSGSSSNIGSNTVHWYQQLPGTAPKLLIYSDNQRPSGVPDRFSGSKSGTSASLAISGLQSEDEADYYCAAWDDSLNGVFGGGTKLTVLGQPKAAPSVTLFPPSSEELQANKATLVCLISDFYPGAVTVAWKADSSPVKAGVETTTPSKQSNNKYAASSYLSLTPEQWKSHRSYSCQVTHEGSTVEKTVAPTECS

SEQ ID NO: 52 - protein, 352 aa, Homo sapiens [sequence omitted]

SEQ ID NO: 53 - protein, 352 aa, Rattus sp.
NEDSEREANVEKEGLCNACAWRQNTRYSRIEAIKIQILSKLRLETAPNISKDAIRQLLPRAPPLRELIDQYDVQRDDSSDGSLEDDDYHATTETIITMPTESDFLMQADGKPKCCFFKFSSKIQYNKVVKAQLWIYLRAVKTPTTVFVQILRLIKPMKDGTRYTGIRSLKLDMSPGTGIWQSIDVKTVLQNWLKQPESNLGIEIKALDENGHDLAVTFPGPGEDGLNPFLEVKVTDTPKRSRRDFGLDCDEHSTESRCCRYPLTVDFEAFGWDWIIAPKRYKANYCSGECEFVFLQKYPHTHLVHQANPRGSAGPCCTPTKMSPINMLYFNGKEQIIYGKIPAMVVDRCGCS

SEQ ID NO: 54 - protein, 352 aa, Mus sp.
NEGSEREENVEKEGLCNACAWRQNTRYSRIEAIKIQILSKLRLETAPNISKDAIRQLLPRAPPLRELIDQYDVQRDDSSDGSLEDDDYHATTETIITMPTESDFLMQADGKPKCCFFKFSSKIQYNKVVKAQLWIYLRPVKTPTTVFVQILRLIKPMKDGTRYTGIRSLKLDMSPGTGIWQSIDVKTVLQNWLKQPESNLGIEIKALDENGHDLAVTFPGPGEDGLNPFLEVKVTDTPKRSRRDFGLDCDEHSTESRCCRYPLTVDFEAFGWDWIIAPKRYKANYCSGECEFVFLQKYPHTHLVHQANPRGSAGPCCTPTKMSPINMLYFNGKEQIIYGKIPAMVVDRCGCS

SEQ ID NO: 55 - protein, 277 aa, Macaca fascicularis
NENSEQKENVEKEGLCNACTWRQNTKSSRIEAIKIQILSKLRLETAPNISKDAIRQLLPKAPPLRELIDQYDVQRDDSSDGSLEDDDYHATTETIITMPTESDFLMQVDGKPKCCFFKFSSKIQYNKVVKAQLWIYLRPVETPTTVFVQILRLIKPMKDGTRYTGIRSLKLDMNPGTGIWQSIDVKTVLQNWLKQPESNLGIEIKALDENGHDLAVTFPGPGEDGLNPFLEVKVTDTPKRSRRDFGLDCDEHSTESRCCRYPLTVDFEAFGWDWIIA

SEQ ID NO: 56 - protein, 109 aa, Unknown
  Description of Unknown: Mature myostatin sequence
DFGLDCDEHSTESRCCRYPLTVDFEAFGWDWIIAPKRYKANYCSGECEFVFLQKYPHTHLVHQANPRGSAGPCCTPTKMSPINMLYFNGKEQIIYGKIPAMVVDRCGCS

SEQ ID NO: 57 - protein, 24 aa, Unknown
  Description of Unknown: Antibody binding epitope sequence
FVQILRLIKPMKDGTRYTGIRSLK

SEQ ID NO: 58 - protein, 5 aa, Artificial Sequence
  Description of Artificial Sequence: Synthetic peptide
CPPCP

SEQ ID NO: 59 - protein, 8 aa, Artificial Sequence
  Description of Artificial Sequence: Synthetic peptide
SSNIGGNT

SEQ ID NO: 60 - protein, 7 aa, Artificial Sequence
  Description of Artificial Sequence: Synthetic peptide
SDNQRPS

SEQ ID NO: 61 - protein, 3 aa, Artificial Sequence
  Description of Artificial Sequence: Synthetic peptide
SDN

SEQ ID NO: 62 - protein, 33 aa, Unknown
  Description of Unknown: Antibody binding sequence
PKAPPLRELIDQYDVQRDDSSDGSLEDDDYHAT

SEQ ID NO: 63 - protein, 34 aa, Unknown
  Description of Unknown: Antibody binding sequence
GLNPFLEVKVTDTPKRSRRDFGLDCDEHSTESRC

SEQ ID NO: 64 - protein, 3 aa, Artificial Sequence
  Description of Artificial Sequence: Synthetic peptide
SDD

SEQ ID NO: 65 - protein, 10 aa, Artificial Sequence
  Description of Artificial Sequence: Synthetic peptide
AAWDDSLNGV

SEQ ID NO: 66 - protein, 5 aa, Artificial Sequence
  Description of Artificial Sequence: Synthetic peptide
SYDIS

SEQ ID NO: 67 - protein, 11 aa, Artificial Sequence
  Description of Artificial Sequence: Synthetic peptide
GVPAYSTGGDL

SEQ ID NO: 68 - protein, 13 aa, Artificial Sequence
  Description of Artificial Sequence: Synthetic peptide
QSSQSVYDNNWLS

SEQ ID NO: 69 - protein, 7 aa, Artificial Sequence
  Description of Artificial Sequence: Synthetic peptide
WASTLAS

SEQ ID NO: 70 - protein, 10 aa, Artificial Sequence
  Description of Artificial Sequence: Synthetic peptide
AGGYGGGLYA

SEQ ID NO: 71 - protein, 17 aa, Artificial Sequence
  Description of Artificial Sequence: Synthetic peptide
ESLIRFLEDPQQGGMDV

SEQ ID NO: 72 - protein, 10 aa, Artificial Sequence
  Description of Artificial Sequence: Synthetic peptide
NSWTRSNNYI

SEQ ID NO: 73 - protein, 126 aa, Artificial Sequence
  Description of Artificial Sequence: Synthetic polypeptide
QVQLQQSGAEVKKPGASVKVSCKASGYTFTSYYMHWVRQAPGQGLEWMGIINPSGGSTSYAQKFQGRVTMTRDTSTSTVYMELSSLRSEDTAVYYCARESLIRFLEDPQQGGMDVWGQGTTVTVSS

SEQ ID NO: 74 - protein, 121 aa, Artificial Sequence
  Description of Artificial Sequence: Synthetic polypeptide
QSALTQPASVSGSPGQSLTISCTGTSSDIGGYNYVSWYQQHPGKAPKLIIYDVTDRPSGVSGRFSGSKSGNTASLTISGLQTEDEAEYFCNSWTRSNNYIFGGGTKLTVLGQPKAAPSVTL

SEQ ID NO: 75 - protein, 273 aa, Artificial Sequence
  Description of Artificial Sequence: Synthetic polypeptide
QVQLQQSGAEVKKPGASVKVSCKASGYTFTSYYMHWVRQAPGQGLEWMGIINPSGGSTSYAQKFQGRVTMTRDTSTSTVYMELSSLRSEDTAVYYCARESLIRFLEDPQQGGMDVWGQGTTVTVSSGSASAPTLGGGGSGGGGSAAAQSALTQPASVSGSPGQSLTISCTGTSSDIGGYNYVSWYQQHPGKAPKLIIYDVTDRPSGVSGRFSGSKSGNTASLTISGLQTEDEAEYFCNSWTRSNNYIFGGGTKLTVLGQPKAAPSVTLFPPSS

SEQ ID NO: 76 - protein, 13 aa, Artificial Sequence
  Description of Artificial Sequence: Synthetic peptide
DRYSSSWGGGFDY

SEQ ID NO: 77 - protein, 10 aa, Artificial Sequence
  Description of Artificial Sequence: Synthetic peptide
QSYDASSLWV

SEQ ID NO: 78 - protein, 122 aa, Artificial Sequence
  Description of Artificial Sequence: Synthetic polypeptide
EVQLVQSGGGVVQSGRSLRLSCVASGFSFSNYGMHWVRQAPGKGLEWLAFIWYDGSNKWYADSVKGRFTISRDNSKNALYLQMNSLRAEDTAVYYCARDRYSSSWGGGFDYWGQGTVLTVSS

SEQ ID NO: 79 - protein, 122 aa, Artificial Sequence
  Description of Artificial Sequence: Synthetic polypeptide
NFMLTQPHSVSESPGRTVTIPCSGRGGSIASDSVQWYQQRPGSAPTTIIYEDNQRPSGVPDRFSGSVDSSSNSASLTISGLRTEDEADYYCQSYDASSLWVFGGKTKLTVLGQPKAAPSVTL

SEQ ID NO: 80 - protein, 275 aa, Artificial Sequence
  Description of Artificial Sequence: Synthetic polypeptide
EVQLVQSGGGVVQSGRSLRLSCVASGFSFSNYGMHWVRQAPGKGLEWLAFIWYDGSNKWYADSVKGRFTISRDNSKNALYLQMNSLRAEDTAVYYCARDRYSSSWGGGFDYWGQGTVLTVSSGSASAPTLGGGGSGGGGSAAANFMLTQPHSVSESPGRTVTIPCSGRGGSIASDSVQWYQQRPGSAPTTIIYEDNQRPSGVPDRFSGSVDSSSNSASLTISGLRTEDEADYYCQSYDASSLWVFGGKTKLTVLGQPKAAPSVTLFPPSSKASGA

SEQ ID NO: 81 - protein, 10 aa, Artificial Sequence
  Description of Artificial Sequence: Synthetic peptide
DRHSLGDFDY

SEQ ID NO: 82 - protein, 9 aa, Artificial Sequence
  Description of Artificial Sequence: Synthetic peptide
QAWDSTTVV

SEQ ID NO: 83 - protein, 121 aa, Artificial Sequence
  Description of Artificial Sequence: Synthetic polypeptide
QLQLQQSGGGLVKPGGSLRLSCAASGFTFSSYSMNWVRQAPGKGLEWVSSISSSSSYIYYADSVKGRFTISRDNAKNSLYLQMNSLRAEDTAVYYCVRDRHSLGDFDYWGQGTLVTVSSGS

SEQ ID NO: 84 - protein, 121 aa, Artificial Sequence
  Description of Artificial Sequence: Synthetic polypeptide
SSELTQPSVSVSPGQTATITCSGDKLGDKYASWYQQKPGQSPVLVIYQDTKRPSGIPARFSGSNSGNTATLTISGTQAMDEAAYYCQAWDSTTVVFGGGTKLTVLGQPKAAPSVTLFPPSS

SEQ ID NO: 85 - protein, 201 aa, Artificial Sequence
  Description of Artificial Sequence: Synthetic polypeptide
QLQLQQSGGGLVKPGGSLRLSCAASGFTFSSYSMNWVRQAPGKGLEWVSSISSSSSYIYYADSVKGRFTISRDNAKNSLYLQMNSLRAEDTAVYYCVRDRHSLGDFDYWGQGTLVTVSSGSASAPTLGGGGSGGGGSAAASSELTQPPSVSVSPGQTATITCSGDKLGDKYASWYQQKPGQSPVLVIYQDTKRPSGIPARF

SEQ ID NO: 86 - protein, 18 aa, Artificial Sequence
  Description of Artificial Sequence: Synthetic peptide
HGLMDDSSGYYLSNAFDI

SEQ ID NO: 87 - protein, 11 aa, Artificial Sequence
  Description of Artificial Sequence: Synthetic peptide
ATWDDSLTGVV

SEQ ID NO: 88 - protein, 129 aa, Artificial Sequence
  Description of Artificial Sequence: Synthetic polypeptide
QVQLVQSGAEVKKPGSSVKVSCKASGGTFSSYAISWVRQAPGQGLEWMGGIIPIFGTANYAQKFQGRVTITADESTSTAYMELSSLRSEDTAVYYCANHGLMDDSSGYYLSNAFDIWGQGTMVTVSSGS

SEQ ID NO: 89 - protein, 126 aa, Artificial Sequence
  Description of Artificial Sequence: Synthetic polypeptide
QPVLTQPPSASGTPGQRVTISCSGSSSNIGSNTVEWYQQLPGTAPKLLIHSNNQRPSGVPDRFSGSRSGTSASLAISGLQSEDEADYFCATWDDSLTGVVFGGGTTLTVLGQPKAAPSVTLFPPSS

SEQ ID NO: 90 - protein, 274 aa, Artificial Sequence
  Description of Artificial Sequence: Synthetic polypeptide
QVQLVQSGAEVKKPGSSVKVSCKASGGTFSSYAISWVRQAPGQGLEWMGGIIPIFGTANYAQKFQGRVTITADESTSTAYMELSSLRSEDTAVYYCANHGLMDDSSGYYLSNAFDIWGQGTMVTVSSGSASAPTLGGGGSGGGGSAAAQPVLTQPPSASGTPGQRVTISCSGSSSNIGSNTVEWYQQLPGTAPKLLIHSNNQRPSGVPDRFSGSRSGTSASLAISGLQSEDEADYFCATWDDSLTGVVFGGGTTLTVLGQPKAAPSVTLFPPSS

SEQ ID NO: 91 - protein, 12 aa, Artificial Sequence
  Description of Artificial Sequence: Synthetic peptide
VGTAAAGDAFDI

SEQ ID NO: 92 - protein, 11 aa, Artificial Sequence
  Description of Artificial Sequence: Synthetic peptide
AAWDDSLSGWV

SEQ ID NO: 93 - protein, 123 aa, Artificial Sequence
  Description of Artificial Sequence: Synthetic polypeptide
QVQLVQSGGGLIQPGGSLRLSCAASGFTVSSYSMNWVRQAPGKGLEWVSYISSSGSTIYYADSVKGRFTISRDNAKNSLYLQMNSLRAEDTALYYCAKVGTAAAGDAFDIWGQGTMVTVSSGS

SEQ ID NO: 94 - protein, 126 aa, Artificial Sequence
  Description of Artificial Sequence: Synthetic polypeptide
QPVLTQPPSASGTPGQRVTISCFGSSSNIGSNYVYWYQQLPGTAPKLLIYRNNQRPSGVPDRFSGSKSGTSASLAISGLRSEDEADYYCAAWDDSLSGWVFGGGTKLTVLGQPKAAPSVTLFPPSS

SEQ ID NO: 95 - protein, 268 aa, Artificial Sequence
  Description of Artificial Sequence: Synthetic polypeptide
QVQLVQSGGGLIQPGGSLRLSCAASGFTVSSYSMNWVRQAPGKGLEWVSYISSSGSTIYYADSVKGRFTISRDNAKNSLYLQMNSLRAEDTALYYCAKVGTAAAGDAFDIWGQGTMVTVSSGSASAPTLGGGGSGGGGSAAAQPVLTQPPSASGTPGQRVTISCFGSSSNIGSNYVYWYQQLPGTAPKLLIYRNNQRPSGVPDRFSGSKSGTSASLAISGLRSEDEADYYCAAWDDSLSGWVFGGGTKLTVLGQPKAAPSVTLFPPSS

SEQ ID NO: 96 - protein, 18 aa, Artificial Sequence
  Description of Artificial Sequence: Synthetic peptide
VGFYDYVWGSYPYDAFDI

SEQ ID NO: 97 - protein, 9 aa, Artificial Sequence
  Description of Artificial Sequence: Synthetic peptide
QQYGTSPLT

SEQ ID NO: 98 - protein, 127 aa, Artificial Sequence
  Description of Artificial Sequence: Synthetic polypeptide
QIQLVQSGAEVKKPGASVKVSCKASGYTFTSYGISWVRQAPGQGLEWMGWISAYNGNTNYAQKLQGRVTMTTDTSTSTAYMELSSLRSEDTAVYYCARVGFYDYVWGSYPYDAFDIWGQGTMVTVSS

SEQ ID NO: 99 - protein, 108 aa, Artificial Sequence
  Description of Artificial Sequence: Synthetic polypeptide
EIVMTQSPGTLSLSPGERATLSCRASQSVSSNYLAWYQQKPGQAPRLLIYDASNRATGIPARFSGSGSGTDFTLTISSLEPEDFALYYCQQYGTSPLTFGGGTKLEIK

SEQ ID NO: 100 - protein, 265 aa, Artificial Sequence
  Description of Artificial Sequence: Synthetic polypeptide
QIQLVQSGAEVKKPGASVKVSCKASGYTFTSYGISWVRQAPGQGLEWMGWISAYNGNTNYAQKLQGRVTMTTDTSTSTAYMELSSLRSEDTAVYYCARVGFYDYVWGSYPYDAFDIWGQGTMVTVSSGSASAPTLGGGGSGGGGSAAAEIVMTQSPGTLSLSPGERATLSCRASQSVSSNYLAWYQQKPGQAPRLLIYDASNRATGIPARFSGSGSGTDFTLTISSLEPEDFALYYCQQYGTSPLTFGGGTKLEIKRTVAAPSVF

SEQ ID NO: 101 - protein, 14 aa, Artificial Sequence
  Description of Artificial Sequence: Synthetic peptide
DTSNGGYSSSSFDY

SEQ ID NO: 102 - protein, 10 aa, Artificial Sequence
  Description of Artificial Sequence: Synthetic peptide
SSYTSSSTLV

SEQ ID NO: 103 - protein, 123 aa, Artificial Sequence
  Description of Artificial Sequence: Synthetic polypeptide
EVQLVQSGGGLVQPGRSLRLSCAASGFTFDDYAMHWVRQAPGKGLEWVSGISWNSGSIGYADSVKGRFTISRDNAKNSLYLQMNSLRAEDTALYYCAKDTSNGGYSSSSFDYWGQGTLVTVSS

SEQ ID NO: 104 - protein, 110 aa, Artificial Sequence
  Description of Artificial Sequence: Synthetic polypeptide
QSALTQPASVSGSPGQSITISCTGTSSDVGGYNYVSWYQQHPGTAPKLMIYDVSYRPSGVSNRFSGSKSGNTASLTISGLQAEDEADYYCSSYTSSSTLVFGTGTKVTVL

SEQ ID NO: 105 - protein, 270 aa, Artificial Sequence
  Description of Artificial Sequence: Synthetic polypeptide
EVQLVQSGGGLVQPGRSLRLSCAASGFTFDDYAMHWVRQAPGKGLEWVSGISWNSGSIGYADSVKGRFTISRDNAKNSLYLQMNSLRAEDTALYYCAKDTSNGGYSSSSFDYWGQGTLVTVSSGSASAPTLGGGGSGGGGSAAAQSALTQPASVSGSPGQSITISCTGTSSDVGGYNYVSWYQQHPGTAPKLMIYDVSYRPSGVSNRFSGSKSGNTASLTISGLQAEDEADYYCSSYTSSSTLVFGTGTKVTVLGQPKANPTVTLFPPSS

SEQ ID NO: 106 - protein, 15 aa, Artificial Sequence
  Description of Artificial Sequence: Synthetic peptide
LVYGGYDEPGYYFDY

SEQ ID NO: 107 - protein, 11 aa, Artificial Sequence
  Description of Artificial Sequence: Synthetic peptide
AAWDDSLNGWV

SEQ ID NO: 108 - protein, 124 aa, Artificial Sequence
  Description of Artificial Sequence: Synthetic polypeptide
EVQLLESRAEVKKPGESLKISCKGSGYSFTSYWIGWVRQMPGKGPEWMGIIYPGDSDTRYSPSFQGQVTISADKSISTAYLQWSSLKASDTAMYYCARLVYGGYDEPGYYFDYWGQGTLVTVSS

SEQ ID NO: 109 - protein, 110 aa, Artificial Sequence
  Description of Artificial Sequence: Synthetic polypeptide
QSVLTQPPSASGTPGQRVTISCSGSSSNIRSNTVNWYQQLPGTAPKLLIYSNNQRPSGVPDRFSGSKSGTSASLAISGLQSEDEADYYCAAWDDSLNGWVFGGGTKLTVL

SEQ ID NO: 110 - protein, 276 aa, Artificial Sequence
  Description of Artificial Sequence: Synthetic polypeptide
EVQLLESRAEVKKPGESLKISCKGSGYSFTSYWIGWVRQMPGKGPEWMGIIYPGDSDTRYSPSFQGQVTISADKSISTAYLQWSSLKASDTAMYYCARLVYGGYDEPGYYFDYWGQGTLVTVSSGSASAPTLGGGGSGGGGSAAAQSVLTQPPSASGTPGQRVTISCSGSSSNIRSNTVNWYQQLPGTAPKLLIYSNNQRPSGVPDRFSGSKSGTSASLAISGLQSEDEADYYCAAWDDSLNGWVFGGGTKLTVLGQPKAAPSVTLFPPSSKASGA

SEQ ID NO: 111 - protein, 14 aa, Artificial Sequence
  Description of Artificial Sequence: Synthetic peptide
VDGLEYSSGHNFDY

SEQ ID NO: 112 - protein, 10 aa, Artificial Sequence
  Description of Artificial Sequence: Synthetic peptide
SSYAGSYTWV

SEQ ID NO: 113 - protein, 123 aa, Artificial Sequence
  Description of Artificial Sequence: Synthetic polypeptide
EVQLVQSGGGLVQPGRSLRLSCAASGFTFDDYAMHWVRQAPGKGLEWVSGISWNSGSIGYADSVKGRFTISRDNSKNTLYLQMNSLRAEDTAVYYCAKVDGLEYSSGHNFDYWGQGTLVTVSS

SEQ ID NO: 114 - protein, 110 aa, Artificial Sequence
  Description of Artificial Sequence: Synthetic polypeptide
QSALTQPPSVSGSPGQSVTISCTGSSSDVGYYDHVSWYQHHPGRAPKVIIYDVTKRPSGVPDRFSGSKSGNTASLTISGLQAEDEADYYCSSYAGSYTWVFGGGTELTVL

SEQ ID NO: 115 - protein, 270 aa, Artificial Sequence
  Description of Artificial Sequence: Synthetic polypeptide
EVQLVQSGGGLVQPGRSLRLSCAASGFTFDDYAMHWVRQAPGKGLEWVSGISWNSGSIGYADSVKGRFTISRDNSKNTLYLQMNSLRAEDTAVYYCAKVDGLEYSSGHNFDYWGQGTLVTVSSGSASAPTLGGGGSGGGGSAAAQSALTQPPSVSGSPGQSVTISCTGSSSDVGYYDHVSWYQHHPGRAPKVIIYDVTKRPSGVPDRFSGSKSGNTASLTISGLQAEDEADYYCSSYAGSYTWVFGGGTELTVLGQPKAAPSVTLFPPSS

SEQ ID NO: 116 - protein, 7 aa, Unknown
  Description of Unknown: GLP-1 analog sequence
EGTFTSD

SEQ ID NO: 117 - protein, 9 aa, Unknown
  Description of Unknown: GLP-1 analog sequence
  MOD_RES (2)..(3): Any amino acid
  MOD_RES (5)..(5): Any amino acid
  MOD_RES (8)..(8): Any amino acid
HXXGXFTXD

SEQ ID NO: 118 - protein, 6 aa, Unknown
  Description of Unknown: Antibody binding epitope sequence
KALDEN

SEQ ID NO: 119 - protein, 5 aa, Artificial Sequence
  Description of Artificial Sequence: Synthetic peptide
HTDIS

SEQ ID NO: 120 - protein, 11 aa, Artificial Sequence
  Description of Artificial Sequence: Synthetic peptide
GVPAYSHGGDL

SEQ ID NO: 121 - protein, 7 aa, Artificial Sequence
  Description of Artificial Sequence: Synthetic peptide
WASTLAY

SEQ ID NO: 122 - protein, 10 aa, Artificial Sequence
  Description of Artificial Sequence: Synthetic peptide
AGGYGGGRYA

SEQ ID NO: 123 - protein, 5 aa, Artificial Sequence
  Description of Artificial Sequence: Synthetic peptide
HDDIS

SEQ ID NO: 124 - protein, 13 aa, Artificial Sequence
  Description of Artificial Sequence: Synthetic peptide
TTSQSVYHENWLS

SEQ ID NO: 125 - protein, 116 aa, Artificial Sequence
  Description of Artificial Sequence: Synthetic polypeptide
QSLEESGGRLVTPGGSLTVTCRVSGIDLSSYDISWVRQAPGKGLEWIGIISYAGSTYYASWAKGRFTISKTSTTVDLKMTSLTTEDTATYFCARGVPAYSTGGDLWGPGTLVTVSS

SEQ ID NO: 126 - protein, 119 aa, Artificial Sequence
  Description of Artificial Sequence: Synthetic polypeptide
QVTLKESGPVLVKPTETLTLTCTVSGIDLSSYDISWVRQAPGKGLEWVGIISYAGSTYYASWAKGRLTISKDTSKNQVVLTMTNMDPVDTATYYCARGVPAYSTGGDLWGQGTLVTVSS

SEQ ID NO: 127 - protein, 119 aa, Artificial Sequence
  Description of Artificial Sequence: Synthetic polypeptide
QVTLKESGPVLVKPTETLTLTCTVSGIDLSHTDISWVRQAPGKGLEWVGIISYAGSTYYASWAKGRLTISKDTSKNQVVLTMTNMDPVDTATYYCARGVPAYSHGGDLWGQGTLVTVSS

SEQ ID NO: 128 - protein, 119 aa, Artificial Sequence
  Description of Artificial Sequence: Synthetic polypeptide
QVQLVESGGGLVQPGGSLRLSCAVSGIDLSHDDISWVRQAPGKGLEWVSIISYAGSTYYASWAKGRLTISKDTSKNQVVLTMTNMDPVDTATYYCARGVPAYSHGGDLWGQGTLVTVSS

SEQ ID NO: 129 - protein, 110 aa, Artificial Sequence
  Description of Artificial Sequence: Synthetic polypeptide
AQVLTQTASSVSAAVGGTVTINCQSSQSVYDNNWLSWFQQKPGQPPKLLIYWASTLASGVPSRFKGSGSGTQFTLTISDLECDDAATYYCAGGYGGGLYAFGGGTKVEIK

SEQ ID NO: 130 - protein, 110 aa, Artificial Sequence
  Description of Artificial Sequence: Synthetic polypeptide
DIVMTQSPATLSLSPGERATLSCTTSQSVYHENWLSWFQQKPGQPPKLLIYWASTLAYGVPSRFSGSGSGTDFTLTISSLQPEDAATYYCAGGYGGGRYAFGQGTKVEIK

SEQ ID NO: 131 - protein, 7 aa, Artificial Sequence
  Description of Artificial Sequence: Synthetic peptide
SDDQRPS

SEQ ID NO: 132 - protein, 110 aa, Artificial Sequence
  Description of Artificial Sequence: Synthetic polypeptide
DIVMTQSPATLSLSPGERATLSCQSSQSVYDNNWLSWFQQKPGQPPKLLIYWASTLASGVPSRFSGSGSGTDFTLTISSLQPEDAATYYCAGGYGGGLYAFGQGTKVEIK

SEQ ID NO: 133 - protein, 110 aa, Artificial sequence
  Description of Artificial Sequence: Synthetic polypeptide
DIVMTQSPATLSLSPGERATLSCTSSQSVYHNNWLSWFQQKPGQPPKLLIYWASTLAYGVPSRFSGSGSGTDFTLTISSLQPEDAATYYCAGGYGGGRYAFGQGTKVEIK